European Patent Specification EP 3 942 038 B1, published September 30, 2026. Title: MODULATORS OF TDP-43. Applicant: ALTERON THERAPEUTICS, LLC. The sequence listing filed with the application follows.

SEQUENCE LISTING (9 sequences)

SEQ ID NO: 1 - DNA, 24 bp, Artificial Sequence
  Description of Artificial Sequence: Synthetic oligonucleotide
tgtgtgtgtgtgtgtgtgtgtgtg

SEQ ID NO: 2 - DNA, 21 bp, Artificial Sequence
  Description of Artificial Sequence: Synthetic oligonucleotide
atggtgtgcttccgcctcttc

SEQ ID NO: 3 - DNA, 24 bp, Artificial Sequence
  Description of Artificial Sequence: Synthetic oligonucleotide
ttacacagactgataaccagtacg

SEQ ID NO: 4 - DNA, 25 bp, Artificial Sequence
  Description of Artificial Sequence: Synthetic oligonucleotide
cagaagtagtgatggagaatgtaac

SEQ ID NO: 5 - DNA, 24 bp, Artificial Sequence
  Description of Artificial Sequence: Synthetic oligonucleotide
gttgacctccactcagtgtgattc

SEQ ID NO: 6 - DNA, 20 bp, Artificial Sequence
  Description of Artificial Sequence: Synthetic oligonucleotide
atgaagctgctcgcagcaac

SEQ ID NO: 7 - DNA, 20 bp, Artificial Sequence
  Description of Artificial Sequence: Synthetic oligonucleotide
tcactgggtggcaggctgtg

SEQ ID NO: 8 - DNA, 20 bp, Artificial Sequence
  Description of Artificial Sequence: Synthetic oligonucleotide
tgctctgaagctcaccaaaa

SEQ ID NO: 9 - DNA, 22 bp, Artificial Sequence
  Description of Artificial Sequence: Synthetic oligonucleotide
ggaacggaagctataccatcat